European Patent Specification EP 3 602 053 B1, published June 28, 2023. Title: METHODS OF ISOLATING NEOANTIGEN-SPECIFIC T CELL RECEPTOR SEQUENCES. Applicant: THE UNITED STATES OF AMERICA, AS REPRESENTED BY THE SECRETARY, DEPARTMENT OF HEALTH AND HUMAN SERVICES. The sequence listing filed with the application follows.

SEQUENCE LISTING (25 sequences)

SEQ ID NO: 1 - protein, 27 aa, Homo sapiens
RAKRSGSGATNFSLLKQAGDVEENPGP

SEQ ID NO: 2 - protein, 25 aa, Homo sapiens
WAKFLDPITGTFHYYHSPTNTVHMY

SEQ ID NO: 3 - protein, 9 aa, Homo sapiens
GADGVGKSA

SEQ ID NO: 4 - protein, 10 aa, Homo sapiens
WSYDSTLLAY

SEQ ID NO: 5 - protein, 24 aa, Homo sapiens
  MISC_FEATURE (2)..(2): Xaa at position 2 is any naturally occurring amino acid
  MISC_FEATURE (4)..(11): Xaa at each of positions 4-11 is any naturally occurring amino acid
  MISC_FEATURE (12)..(23): Xaa at each of positions 12-23 is no amino acid or is any naturally occurring amino acid
  MISC_FEATURE (24)..(24): Xaa at position 24 is phenylalanine or tryptophan
YXCXXXXXXXXXXXXXXXXXXXXX

SEQ ID NO: 6 - DNA, 39 bp, Homo sapiens
tgtgctgtgagagaccatagcaactatcagttaatctgg

SEQ ID NO: 7 - protein, 13 aa, Homo sapiens
CAVRDHSNYQLIW

SEQ ID NO: 8 - DNA, 54 bp, Homo sapiens
tgtgccagcagccaatccggtgggggcgggttctcctacaatgagcagttcttc

SEQ ID NO: 9 - protein, 18 aa, Homo sapiens
CASSQSGGGGFSYNEQFF

SEQ ID NO: 10 - DNA, 45 bp, Homo sapiens
tgcctcgtgggtgacatggaccaggcaggaactgctctgatcttt

SEQ ID NO: 11 - protein, 15 aa, Homo sapiens
CLVGDMDQAGTALIF

SEQ ID NO: 12 - DNA, 45 bp, Homo sapiens
tgtgccagcagcttggggagggcaagcaatcagccccagcatttt

SEQ ID NO: 13 - protein, 15 aa, Homo sapiens
CASSLGRASNQPQHF

SEQ ID NO: 14 - DNA, 39 bp, Homo sapiens
tgtgctttcatgtggggattaggtcagaattttgtcttt

SEQ ID NO: 15 - protein, 13 aa, Homo sapiens
CAFMWGLGQNFVF

SEQ ID NO: 16 - DNA, 45 bp, Homo sapiens
tgtgccagcagtgtggagcgggagaacaccggggagctgtttttt

SEQ ID NO: 17 - protein, 15 aa, Homo sapiens
CASSVERENTGELFF

SEQ ID NO: 18 - protein, 14 aa, Homo sapiens
VWDALFADGLSLCL

SEQ ID NO: 19 - protein, 13 aa, Homo sapiens
WRRVAWSYDSTLL

SEQ ID NO: 20 - protein, 8 aa, Homo sapiens
WSYDSTLL

SEQ ID NO: 21 - protein, 9 aa, Homo sapiens
WSYDSTLLA

SEQ ID NO: 22 - protein, 10 aa, Homo sapiens
WSYDSTLLAY

SEQ ID NO: 23 - protein, 12 aa, Homo sapiens
YLALVDKNIIGY

SEQ ID NO: 24 - protein, 9 aa, Homo sapiens
YSEPDVSGK

SEQ ID NO: 25 - protein, 25 aa, Homo sapiens
LGKFPELFNWFKIFLGYKESVHLET